European Patent Application EP 4 610 652 A1, published September 3, 2025. Title: YaxAB nanopore, nanopore system comprising the same and applications thereof. Applicant: Korea Research Institute of Bioscience and Biotechnology. Application KR. The sequence listing filed with the application follows.

SEQUENCE LISTING (36 sequences)

SEQ ID NO: 1 - protein, 366 aa, synthetic construct
IFTKEDLINLKLYVRKGLSLPTRQDEVEAYLGYKKIDVAGLEPKDIKLLFDEIHNHALNWNDVEQAVLQQSLDLDIAAKNIISTGNEIINLINQMPITLRVKTLLGDITDKQLENITYESADHEVASALKDILDDMKGDINRHQTTTENVRKKVSDYRITLTGGELSSGDKVNGLEPQVKTKYDLMEKSNMRKSIKELDEKIKEKRQRIEQLKKDYDKFVGLSFTGAIGGIIAMAITGGIFGAKAENARKEKNALISEVAELESKVSSQRALQTALEALSLSFSDIGIRMVDAESALNHLDFMWLSVLNQITESQIQFAMINNALRLTSFVNKFQQVITPWQSVGDSARQLVDIFDEAIKEYKKVY

SEQ ID NO: 2 - protein, 332 aa, synthetic construct
LSYPDINFKIFSQGVKNISHLAQFKTTGVEVLQEKALRVSLYSQRLDVIVRESLSSLQVKLENTLALTYFTTLEEIDEALISQDIDEESKSEMRKERINIIKNLSNDITQLKQLFIEKTELLDKSSSDLHNVVIIEGTDKVLQAEQLRQKQLTEDIATKELERKEIEKKRDKIIEALDVIREHNLVDAFKDLIPTGENLSELDLAKPEIELLKQSLEITKKLLGQFSEGLKYIDLTDARKKLDNQIDTASTRLTELNRQLEQSEKLIAGVNAVIKIDQEKSAVVVEAEKLSRAWHIFIHEITALQGTSLNEVELSKPLIKQQIYLESLIKQL

SEQ ID NO: 3 - protein, 411 aa, synthetic construct
MTQTQLAIDNVLASAESTIQLNELPKVVLDFITGEQTSVARSGGIFTKEDLINLKLYVRKGLSLPTRQDEVEAYLGYKKIDVAGLEPKDIKLLFDEIHNHALNWNDVEQAVLQQSLDLDIAAKNIISTGNEIINLINQMPITLRVKTLLGDITDKQLENITYESADHEVASALKDILDDMKGDINRHQTTTENVRKKVSDYRITLTGGELSSGDKVNGLEPQVKTKYDLMEKSNMRKSIKELDEKIKEKRQRIEQLKKDYDKFVGLSFTGAIGGIIAMAITGGIFGAKAENARKEKNALISEVAELESKVSSQRALQTALEALSLSFSDIGIRMVDAESALNHLDFMWLSVLNQITESQIQFAMINNALRLTSFVNKFQQVITPWQSVGDSARQLVDIFDEAIKEYKKVYG

SEQ ID NO: 4 - protein, 344 aa, synthetic construct
MAEISTFPHSGLSYPDINFKIFSQGVKNISHLAQFKTTGVEVLQEKALRVSLYSQRLDVIVRESLSSLQVKLENTLALTYFTTLEEIDEALISQDIDEESKSEMRKERINIIKNLSNDITQLKQLFIEKTELLDKSSSDLHNVVIIEGTDKVLQAEQLRQKQLTEDIATKELERKEIEKKRDKIIEALDVIREHNLVDAFKDLIPTGENLSELDLAKPEIELLKQSLEITKKLLGQFSEGLKYIDLTDARKKLDNQIDTASTRLTELNRQLEQSEKLIAGVNAVIKIDQEKSAVVVEAEKLSRAWHIFIHEITALQGTSLNEVELSKPLIKQQIYLESLIKQLI

SEQ ID NO: 5 - protein, 361 aa, synthetic construct
LINLKLYVRKGLSLPTRQDEVEAYLGYKKIDVAGLEPKDIKLLFDEIHNHALNWNDVEQAVLQQSLDLDIAAKNIISTGNEIINLINQMPITLRVKTLLGDITDKQLENITYESADHEVASALKDILDDMKGDINRHQTTTENVRKKVSDYRITLTGGELSSGDKVNGLEPQVKTKYDLMEKSNMRKSIKELDEKIKEKRQRIEQLKKDYDKFVGLSFTGAIGGIIAMAITGGIFGAKAENARKEKNALISEVAELESKVSSQRALQTALEALSLSFSDIGIRMVDAESALNHLDFMWLSVLNQITESQIQFAMINNALRLTSFVNKFQQVITPWQSVGDSARQLVDIFDEAIKEYKKVYG

SEQ ID NO: 6 - protein, 408 aa, synthetic construct
QTQLAIDNVLASAESTIQLNELPKVVLDFITGEQTSVARSGGIFTKEDLINLKLYVRKGLSLPTRQDEVEAYLGYKKIDVAGLEPKDIKLLFDEIHNHALNWNDVEQAVLQQSLDLDIAAKNIISTGNEIINLINQMPITLRVKTLLGDITDKQLENITYESADHEVASALKDILDDMKGDINRHQTTTENVRKKVSDYRITLTGGELSSGDKVNGLEPQVKTKYDLMEKSNMRKSIKELDEKIKEKRQRIEQLKKDYDKFVGLSFTGAIGGIIAMAITGGIFGAKAENARKEKNALISEVAELESKVSSQRALQTALEALSLSFSDIGIRMVDAESALNHLDFMWLSVLNQITESQIQFAMINNALRLTSFVNKFQQVITPWQSVGDSARQLVDIFDEAIKEYKKVY

SEQ ID NO: 7 - protein, 342 aa, synthetic construct
YVRKGLSLPTRQDEVEAYLGYKKIDVAGLEPKDIKLLFDEIHNHALNWNDVEQAVLQQSLDLDIAAKNIISTGNEIINLINQMPITLRVKTLLGDITDKQLENITYESADHEVASALKDILDDMKGDINRHQTTTENVRKKVSDYRITLTGGELSSGDKVNGLEPQVKTKYDLMEKSNMRKSIKELDEKIKEKRQRIEQLKKDYDKFVGLSFTGAIGGIIAMAITGGIFGAKAENARKEKNALISEVAELESKVSSQRALQTALEALSLSFSDIGIRMVDAESALNHLDFMWLSVLNQITESQIQFAMINNALRLTSFVNKFQQVITPWQSVGDSARQLVDI

SEQ ID NO: 8 - protein, 406 aa, synthetic construct
QLAIDNVLASAESTIQLNELPKVVLDFITGEQTSVARSGGIFTKEDLINLKLYVRKGLSLPTRQDEVEAYLGYKKIDVAGLEPKDIKLLFDEIHNHALNWNDVEQAVLQQSLDLDIAAKNIISTGNEIINLINQMPITLRVKTLLGDITDKQLENITYESADHEVASALKDILDDMKGDINRHQTTTENVRKKVSDYRITLTGGELSSGDKVNGLEPQVKTKYDLMEKSNMRKSIKELDEKIKEKRQRIEQLKKDYDKFVGLSFTGAIGGIIAMAITGGIFGAKAENARKEKNALISEVAELESKVSSQRALQTALEALSLSFSDIGIRMVDAESALNHLDFMWLSVLNQITESQIQFAMINNALRLTSFVNKFQQVITPWQSVGDSARQLVDIFDEAIKEYKKVY

SEQ ID NO: 9 - protein, 401 aa, synthetic construct
VLASAESTIQLNELPKVVLDFITGEQTSVARSGGIFTKEDLINLKLYVRKGLSLPTRQDEVEAYLGYKKIDVAGLEPKDIKLLFDEIHNHALNWNDVEQAVLQQSLDLDIAAKNIISTGNEIINLINQMPITLRVKTLLGDITDKQLENITYESADHEVASALKDILDDMKGDINRHQTTTENVRKKVSDYRITLTGGELSSGDKVNGLEPQVKTKYDLMEKSNMRKSIKELDEKIKEKRQRIEQLKKDYDKFVGLSFTGAIGGIIAMAITGGIFGAKAENARKEKNALISEVAELESKVSSQRALQTALEALSLSFSDIGIRMVDAESALNHLDFMWLSVLNQITESQIQFAMINNALRLTSFVNKFQQVITPWQSVGDSARQLVDIFDEAIKEYKKVYG

SEQ ID NO: 10 - protein, 391 aa, synthetic construct
LNELPKVVLDFITGEQTSVARSGGIFTKEDLINLKLYVRKGLSLPTRQDEVEAYLGYKKIDVAGLEPKDIKLLFDEIHNHALNWNDVEQAVLQQSLDLDIAAKNIISTGNEIINLINQMPITLRVKTLLGDITDKQLENITYESADHEVASALKDILDDMKGDINRHQTTTENVRKKVSDYRITLTGGELSSGDKVNGLEPQVKTKYDLMEKSNMRKSIKELDEKIKEKRQRIEQLKKDYDKFVGLSFTGAIGGIIAMAITGGIFGAKAENARKEKNALISEVAELESKVSSQRALQTALEALSLSFSDIGIRMVDAESALNHLDFMWLSVLNQITESQIQFAMINNALRLTSFVNKFQQVITPWQSVGDSARQLVDIFDEAIKEYKKVYG

SEQ ID NO: 11 - protein, 381 aa, synthetic construct
FITGEQTSVARSGGIFTKEDLINLKLYVRKGLSLPTRQDEVEAYLGYKKIDVAGLEPKDIKLLFDEIHNHALNWNDVEQAVLQQSLDLDIAAKNIISTGNEIINLINQMPITLRVKTLLGDITDKQLENITYESADHEVASALKDILDDMKGDINRHQTTTENVRKKVSDYRITLTGGELSSGDKVNGLEPQVKTKYDLMEKSNMRKSIKELDEKIKEKRQRIEQLKKDYDKFVGLSFTGAIGGIIAMAITGGIFGAKAENARKEKNALISEVAELESKVSSQRALQTALEALSLSFSDIGIRMVDAESALNHLDFMWLSVLNQITESQIQFAMINNALRLTSFVNKFQQVITPWQSVGDSARQLVDIFDEAIKEYKKVYG

SEQ ID NO: 12 - protein, 371 aa, synthetic construct
RSGGIFTKEDLINLKLYVRKGLSLPTRQDEVEAYLGYKKIDVAGLEPKDIKLLFDEIHNHALNWNDVEQAVLQQSLDLDIAAKNIISTGNEIINLINQMPITLRVKTLLGDITDKQLENITYESADHEVASALKDILDDMKGDINRHQTTTENVRKKVSDYRITLTGGELSSGDKVNGLEPQVKTKYDLMEKSNMRKSIKELDEKIKEKRQRIEQLKKDYDKFVGLSFTGAIGGIIAMAITGGIFGAKAENARKEKNALISEVAELESKVSSQRALQTALEALSLSFSDIGIRMVDAESALNHLDFMWLSVLNQITESQIQFAMINNALRLTSFVNKFQQVITPWQSVGDSARQLVDIFDEAIKEYKKVYG

SEQ ID NO: 13 - protein, 354 aa, synthetic construct
YVRKGLSLPTRQDEVEAYLGYKKIDVAGLEPKDIKLLFDEIHNHALNWNDVEQAVLQQSLDLDIAAKNIISTGNEIINLINQMPITLRVKTLLGDITDKQLENITYESADHEVASALKDILDDMKGDINRHQTTTENVRKKVSDYRITLTGGELSSGDKVNGLEPQVKTKYDLMEKSNMRKSIKELDEKIKEKRQRIEQLKKDYDKFVGLSFTGAIGGIIAMAITGGIFGAKAENARKEKNALISEVAELESKVSSQRALQTALEALSLSFSDIGIRMVDAESALNHLDFMWLSVLNQITESQIQFAMINNALRLTSFVNKFQQVITPWQSVGDSARQLVDIFDEAIKEYKKVY

SEQ ID NO: 14 - protein, 355 aa, synthetic construct
LYVRKGLSLPTRQDEVEAYLGYKKIDVAGLEPKDIKLLFDEIHNHALNWNDVEQAVLQQSLDLDIAAKNIISTGNEIINLINQMPITLRVKTLLGDITDKQLENITYESADHEVASALKDILDDMKGDINRHQTTTENVRKKVSDYRITLTGGELSSGDKVNGLEPQVKTKYDLMEKSNMRKSIKELDEKIKEKRQRIEQLKKDYDKFVGLSFTGAIGGIIAMAITGGIFGAKAENARKEKNALISEVAELESKVSSQRALQTALEALSLSFSDIGIRMVDAESALNHLDFMWLSVLNQITESQIQFAMINNALRLTSFVNKFQQVITPWQSVGDSARQLVDIFDEAIKEYKKVY

SEQ ID NO: 15 - protein, 343 aa, synthetic construct
YVRKGLSLPTRQDEVEAYLGYKKIDVAGLEPKDIKLLFDEIHNHALNWNDVEQAVLQQSLDLDIAAKNIISTGNEIINLINQMPITLRVKTLLGDITDKQLENITYESADHEVASALKDILDDMKGDINRHQTTTENVRKKVSDYRITLTGGELSSGDKVNGLEPQVKTKYDLMEKSNMRKSIKELDEKIKEKRQRIEQLKKDYDKFVGLSFTGAIGGIIAMAITGGIFGAKAENARKEKNALISEVAELESKVSSQRALQTALEALSLSFSDIGIRMVDAESALNHLDFMWLSVLNQITESQIQFAMINNALRLTSFVNKFQQVITPWQSVGDSARQLVDIF

SEQ ID NO: 16 - protein, 345 aa, synthetic construct
YVRKGLSLPTRQDEVEAYLGYKKIDVAGLEPKDIKLLFDEIHNHALNWNDVEQAVLQQSLDLDIAAKNIISTGNEIINLINQMPITLRVKTLLGDITDKQLENITYESADHEVASALKDILDDMKGDINRHQTTTENVRKKVSDYRITLTGGELSSGDKVNGLEPQVKTKYDLMEKSNMRKSIKELDEKIKEKRQRIEQLKKDYDKFVGLSFTGAIGGIIAMAITGGIFGAKAENARKEKNALISEVAELESKVSSQRALQTALEALSLSFSDIGIRMVDAESALNHLDFMWLSVLNQITESQIQFAMINNALRLTSFVNKFQQVITPWQSVGDSARQLVDIFDE

SEQ ID NO: 17 - protein, 348 aa, synthetic construct
YVRKGLSLPTRQDEVEAYLGYKKIDVAGLEPKDIKLLFDEIHNHALNWNDVEQAVLQQSLDLDIAAKNIISTGNEIINLINQMPITLRVKTLLGDITDKQLENITYESADHEVASALKDILDDMKGDINRHQTTTENVRKKVSDYRITLTGGELSSGDKVNGLEPQVKTKYDLMEKSNMRKSIKELDEKIKEKRQRIEQLKKDYDKFVGLSFTGAIGGIIAMAITGGIFGAKAENARKEKNALISEVAELESKVSSQRALQTALEALSLSFSDIGIRMVDAESALNHLDFMWLSVLNQITESQIQFAMINNALRLTSFVNKFQQVITPWQSVGDSARQLVDIFDEAIK

SEQ ID NO: 18 - protein, 317 aa, synthetic construct
VKNISHLAQFKTTGVEVLQEKALRVSLYSQRLDVIVRESLSSLQVKLENTLALTYFTTLEEIDEALISQDIDEESKSEMRKERINIIKNLSNDITQLKQLFIEKTELLDKSSSDLHNVVIIEGTDKVLQAEQLRQKQLTEDIATKELERKEIEKKRDKIIEALDVIREHNLVDAFKDLIPTGENLSELDLAKPEIELLKQSLEITKKLLGQFSEGLKYIDLTDARKKLDNQIDTASTRLTELNRQLEQSEKLIAGVNAVIKIDQEKSAVVVEAEKLSRAWHIFIHEITALQGTSLNEVELSKPLIKQQIYLESLIKQ

SEQ ID NO: 19 - protein, 339 aa, synthetic construct
IFTKEDLINLKLYVRKGLSLPTRQDEVEAYLGYKKIDVAGLEPKDIKLLFDEIHNHALNWNDVEQAVLQQSLDLDIAAKNIISTGNEIINLINQMPITLRVKTLLGDITDKQLENITYESADHEVASALKDILDDMKGDINRHQTTTENVRKKVSDYRITLTGGELSSGDKVNGLEPQVKTKYDLMEKSNMRKSIKELDEKIKEKRQRIEQLKKDYDKFVGLSFTGAIGGIIAMAITGGIFGAKAENARKEKNALISEVAELESKVSSQRALQTALEALSLSFSDIGIRMVDAESALNHLDFMWLSVLNQITESQIQFAMINNALRLTSFVNKFQQVIT

SEQ ID NO: 20 - protein, 341 aa, synthetic construct
IFTKEDLINLKLYVRKGLSLPTRQDEVEAYLGYKKIDVAGLEPKDIKLLFDEIHNHALNWNDVEQAVLQQSLDLDIAAKNIISTGNEIINLINQMPITLRVKTLLGDITDKQLENITYESADHEVASALKDILDDMKGDINRHQTTTENVRKKVSDYRITLTGGELSSGDKVNGLEPQVKTKYDLMEKSNMRKSIKELDEKIKEKRQRIEQLKKDYDKFVGLSFTGAIGGIIAMAITGGIFGAKAENARKEKNALISEVAELESKVSSQRALQTALEALSLSFSDIGIRMVDAESALNHLDFMWLSVLNQITESQIQFAMINNALRLTSFVNKFQQVITPW

SEQ ID NO: 21 - protein, 343 aa, synthetic construct
IFTKEDLINLKLYVRKGLSLPTRQDEVEAYLGYKKIDVAGLEPKDIKLLFDEIHNHALNWNDVEQAVLQQSLDLDIAAKNIISTGNEIINLINQMPITLRVKTLLGDITDKQLENITYESADHEVASALKDILDDMKGDINRHQTTTENVRKKVSDYRITLTGGELSSGDKVNGLEPQVKTKYDLMEKSNMRKSIKELDEKIKEKRQRIEQLKKDYDKFVGLSFTGAIGGIIAMAITGGIFGAKAENARKEKNALISEVAELESKVSSQRALQTALEALSLSFSDIGIRMVDAESALNHLDFMWLSVLNQITESQIQFAMINNALRLTSFVNKFQQVITPWQS

SEQ ID NO: 22 - protein, 345 aa, synthetic construct
IFTKEDLINLKLYVRKGLSLPTRQDEVEAYLGYKKIDVAGLEPKDIKLLFDEIHNHALNWNDVEQAVLQQSLDLDIAAKNIISTGNEIINLINQMPITLRVKTLLGDITDKQLENITYESADHEVASALKDILDDMKGDINRHQTTTENVRKKVSDYRITLTGGELSSGDKVNGLEPQVKTKYDLMEKSNMRKSIKELDEKIKEKRQRIEQLKKDYDKFVGLSFTGAIGGIIAMAITGGIFGAKAENARKEKNALISEVAELESKVSSQRALQTALEALSLSFSDIGIRMVDAESALNHLDFMWLSVLNQITESQIQFAMINNALRLTSFVNKFQQVITPWQSVG

SEQ ID NO: 23 - protein, 346 aa, synthetic construct
IFTKEDLINLKLYVRKGLSLPTRQDEVEAYLGYKKIDVAGLEPKDIKLLFDEIHNHALNWNDVEQAVLQQSLDLDIAAKNIISTGNEIINLINQMPITLRVKTLLGDITDKQLENITYESADHEVASALKDILDDMKGDINRHQTTTENVRKKVSDYRITLTGGELSSGDKVNGLEPQVKTKYDLMEKSNMRKSIKELDEKIKEKRQRIEQLKKDYDKFVGLSFTGAIGGIIAMAITGGIFGAKAENARKEKNALISEVAELESKVSSQRALQTALEALSLSFSDIGIRMVDAESALNHLDFMWLSVLNQITESQIQFAMINNALRLTSFVNKFQQVITPWQSVGD

SEQ ID NO: 24 - protein, 332 aa, synthetic construct
INLKLYVRKGLSLPTRQDEVEAYLGYKKIDVAGLEPKDIKLLFDEIHNHALNWNDVEQAVLQQSLDLDIAAKNIISTGNEIINLINQMPITLRVKTLLGDITDKQLENITYESADHEVASALKDILDDMKGDINRHQTTTENVRKKVSDYRITLTGGELSSGDKVNGLEPQVKTKYDLMEKSNMRKSIKELDEKIKEKRQRIEQLKKDYDKFVGLSFTGAIGGIIAMAITGGIFGAKAENARKEKNALISEVAELESKVSSQRALQTALEALSLSFSDIGIRMVDAESALNHLDFMWLSVLNQITESQIQFAMINNALRLTSFVNKFQQVIT

SEQ ID NO: 25 - protein, 305 aa, synthetic construct
LSYPDINFKIFSQGVKNISHLAQFKTTGVEVLQEKALRVSLYSQRLDVIVRESLSSLQVKLENTLALTYFTTLEEIDEALISQDIDEESKSEMRKERINIIKNLSNDITQLKQLFIEKTELLDKSSSDLHNVVIIEGTDKVLQAEQLRQKQLTEDIATKELERKEIEKKRDKIIEALDVIREHNLVDAFKDLIPTGENLSELDLAKPEIELLKQSLEITKKLLGQFSEGLKYIDLTDARKKLDNQIDTASTRLTELNRQLEQSEKLIAGVNAVIKIDQEKSAVVVEAEKLSRAWHIFIHEITALQ

SEQ ID NO: 26 - protein, 307 aa, synthetic construct
LSYPDINFKIFSQGVKNISHLAQFKTTGVEVLQEKALRVSLYSQRLDVIVRESLSSLQVKLENTLALTYFTTLEEIDEALISQDIDEESKSEMRKERINIIKNLSNDITQLKQLFIEKTELLDKSSSDLHNVVIIEGTDKVLQAEQLRQKQLTEDIATKELERKEIEKKRDKIIEALDVIREHNLVDAFKDLIPTGENLSELDLAKPEIELLKQSLEITKKLLGQFSEGLKYIDLTDARKKLDNQIDTASTRLTELNRQLEQSEKLIAGVNAVIKIDQEKSAVVVEAEKLSRAWHIFIHEITALQGT

SEQ ID NO: 27 - protein, 308 aa, synthetic construct
LSYPDINFKIFSQGVKNISHLAQFKTTGVEVLQEKALRVSLYSQRLDVIVRESLSSLQVKLENTLALTYFTTLEEIDEALISQDIDEESKSEMRKERINIIKNLSNDITQLKQLFIEKTELLDKSSSDLHNVVIIEGTDKVLQAEQLRQKQLTEDIATKELERKEIEKKRDKIIEALDVIREHNLVDAFKDLIPTGENLSELDLAKPEIELLKQSLEITKKLLGQFSEGLKYIDLTDARKKLDNQIDTASTRLTELNRQLEQSEKLIAGVNAVIKIDQEKSAVVVEAEKLSRAWHIFIHEITALQGTS

SEQ ID NO: 28 - protein, 311 aa, synthetic construct
LSYPDINFKIFSQGVKNISHLAQFKTTGVEVLQEKALRVSLYSQRLDVIVRESLSSLQVKLENTLALTYFTTLEEIDEALISQDIDEESKSEMRKERINIIKNLSNDITQLKQLFIEKTELLDKSSSDLHNVVIIEGTDKVLQAEQLRQKQLTEDIATKELERKEIEKKRDKIIEALDVIREHNLVDAFKDLIPTGENLSELDLAKPEIELLKQSLEITKKLLGQFSEGLKYIDLTDARKKLDNQIDTASTRLTELNRQLEQSEKLIAGVNAVIKIDQEKSAVVVEAEKLSRAWHIFIHEITALQGTSLNE

SEQ ID NO: 29 - protein, 314 aa, synthetic construct
LSYPDINFKIFSQGVKNISHLAQFKTTGVEVLQEKALRVSLYSQRLDVIVRESLSSLQVKLENTLALTYFTTLEEIDEALISQDIDEESKSEMRKERINIIKNLSNDITQLKQLFIEKTELLDKSSSDLHNVVIIEGTDKVLQAEQLRQKQLTEDIATKELERKEIEKKRDKIIEALDVIREHNLVDAFKDLIPTGENLSELDLAKPEIELLKQSLEITKKLLGQFSEGLKYIDLTDARKKLDNQIDTASTRLTELNRQLEQSEKLIAGVNAVIKIDQEKSAVVVEAEKLSRAWHIFIHEITALQGTSLNEVEL

SEQ ID NO: 30 - protein, 403 aa, synthetic construct
IDNVLASAESTIQLNELPKVVLDFITGEQTSVARSGGIFTKEDLINLKLYVRKGLSLPTRQDEVEAYLGYKKIDVAGLEPKDIKLLFDEIHNHALNWNDVEQAVLQQSLDLDIAAKNIISTGNEIINLINQMPITLRVKTLLGDITDKQLENITYESADHEVASALKDILDDMKGDINRHQTTTENVRKKVSDYRITLTGGELSSGDKVNGLEPQVKTKYDLMEKSNMRKSIKELDEKIKEKRQRIEQLKKDYDKFVGLSFTGAIGGIIAMAITGGIFGAKAENARKEKNALISEVAELESKVSSQRALQTALEALSLSFSDIGIRMVDAESALNHLDFMWLSVLNQITESQIQFAMINNALRLTSFVNKFQQVITPWQSVGDSARQLVDIFDEAIKEYKKVY

SEQ ID NO: 31 - protein, 402 aa, synthetic construct
DNVLASAESTIQLNELPKVVLDFITGEQTSVARSGGIFTKEDLINLKLYVRKGLSLPTRQDEVEAYLGYKKIDVAGLEPKDIKLLFDEIHNHALNWNDVEQAVLQQSLDLDIAAKNIISTGNEIINLINQMPITLRVKTLLGDITDKQLENITYESADHEVASALKDILDDMKGDINRHQTTTENVRKKVSDYRITLTGGELSSGDKVNGLEPQVKTKYDLMEKSNMRKSIKELDEKIKEKRQRIEQLKKDYDKFVGLSFTGAIGGIIAMAITGGIFGAKAENARKEKNALISEVAELESKVSSQRALQTALEALSLSFSDIGIRMVDAESALNHLDFMWLSVLNQITESQIQFAMINNALRLTSFVNKFQQVITPWQSVGDSARQLVDIFDEAIKEYKKVY

SEQ ID NO: 32 - protein, 351 aa, synthetic construct
GLSLPTRQDEVEAYLGYKKIDVAGLEPKDIKLLFDEIHNHALNWNDVEQAVLQQSLDLDIAAKNIISTGNEIINLINQMPITLRVKTLLGDITDKQLENITYESADHEVASALKDILDDMKGDINRHQTTTENVRKKVSDYRITLTGGELSSGDKVNGLEPQVKTKYDLMEKSNMRKSIKELDEKIKEKRQRIEQLKKDYDKFVGLSFTGAIGGIIAMAITGGIFGAKAENARKEKNALISEVAELESKVSSQRALQTALEALSLSFSDIGIRMVDAESALNHLDFMWLSVLNQITESQIQFAMINNALRLTSFVNKFQQVITPWQSVGDSARQLVDIFDEAIKEYKKVYG

SEQ ID NO: 33 - protein, 341 aa, synthetic construct
VEAYLGYKKIDVAGLEPKDIKLLFDEIHNHALNWNDVEQAVLQQSLDLDIAAKNIISTGNEIINLINQMPITLRVKTLLGDITDKQLENITYESADHEVASALKDILDDMKGDINRHQTTTENVRKKVSDYRITLTGGELSSGDKVNGLEPQVKTKYDLMEKSNMRKSIKELDEKIKEKRQRIEQLKKDYDKFVGLSFTGAIGGIIAMAITGGIFGAKAENARKEKNALISEVAELESKVSSQRALQTALEALSLSFSDIGIRMVDAESALNHLDFMWLSVLNQITESQIQFAMINNALRLTSFVNKFQQVITPWQSVGDSARQLVDIFDEAIKEYKKVYG

SEQ ID NO: 34 - protein, 331 aa, synthetic construct
DVAGLEPKDIKLLFDEIHNHALNWNDVEQAVLQQSLDLDIAAKNIISTGNEIINLINQMPITLRVKTLLGDITDKQLENITYESADHEVASALKDILDDMKGDINRHQTTTENVRKKVSDYRITLTGGELSSGDKVNGLEPQVKTKYDLMEKSNMRKSIKELDEKIKEKRQRIEQLKKDYDKFVGLSFTGAIGGIIAMAITGGIFGAKAENARKEKNALISEVAELESKVSSQRALQTALEALSLSFSDIGIRMVDAESALNHLDFMWLSVLNQITESQIQFAMINNALRLTSFVNKFQQVITPWQSVGDSARQLVDIFDEAIKEYKKVYG

SEQ ID NO: 35 - protein, 411 aa, synthetic construct
MTQTQLAIDNVLASAENTIQLNELPKVVLDFITGEQTSVARSGGIFTKEDLINLKLYVRKGLSLPTRQDEVEAYLGYKKIDVAGLEPKDIKLLFDEIHNHALNWNDVEQAVLQQSLDLDIAAKNIISTGNEIINLINQMPITLRVKTLLRDITDKQLENITYESADHEVASALKDILDDMKGDINRHQTTTENVRKKVSDYRITLTGGELSSGDKVNGLEPQVKTKYDLMEKSNMRKSIKELDEKIKEKKQRIEQLKKDYDKFVGLSFTGAIGGIIAMAITSGIFGAKAENARKEKNALISEVAELESKVSSQRALQTALEALSLSFSDIGIRMVDAESALNHLDFMWLSVLNQITESQIQFAMINNALRLTSFVNKFQQVITPWQSVGDSARQLVDIFDEAIKEYKKVYG

SEQ ID NO: 36 - protein, 344 aa, synthetic construct
MAEISTFPHSGLSYPDINFKIFSQGVKNISHLAQFKTTGVEVLQEKALRVSLYSQRLDVIVRESLSSLQVKLENTLALTYFTTLEEIDEALISQDIDEESKSEMRKERINIIKNLSNDITQLKQLFIEKTELLDKSSSDLHNVVIIEGTDKVLQAEQLRQKQLTEDIATKELERKEIEKKRDKIIEALDVIREHNLVDAFKDLIPTGENLSELDLAKPEIELLKQSLEITKKLLGQFSEGLKYIDLTDARKKLDNQIDTASTRLTELNRQLEQSEKLIAGVNAIIKIDQEKSAVVVEAEKLSRAWHIFIHEITALQGTSLNEVELSKPLIKQQIYLESLIKQLI